European Patent Specification EP 3 797 170 B1, published July 19, 2023. Title: POLYNUCLEOTIDE SYNTHESIS METHOD, SYSTEM AND KIT. Applicant: OXFORD NANOPORE TECHNOLOGIES LIMITED. Application To be assigned. The sequence listing filed with the application follows.

SEQUENCE LISTING (69 sequences)

SEQ ID NO: 1 - DNA, 18 bp, Artificial Sequence
  source: /note="Description of Artificial Sequence: Synthetic primer"
gcgacaggtgactgcagc

SEQ ID NO: 2 - DNA, 36 bp, Artificial Sequence
  source: /note="Description of Artificial Sequence: Synthetic oligonucleotide"
  modified_base (18)..(18): 2'-deoxyinosine
cacatcacgtcgtagtcngctgcagtcacctgtcgc

SEQ ID NO: 3 - DNA, 36 bp, Artificial Sequence; identical to SEQ ID NO: 2
  source: /note="Description of Artificial Sequence: Synthetic oligonucleotide"
  modified_base (18)..(18): 2'-deoxyinosine

SEQ ID NO: 4 - DNA, 19 bp, Artificial Sequence
  source: /note="Description of Artificial Sequence: Synthetic primer"
gcgacaggtgactgcagct

SEQ ID NO: 5 - DNA, 36 bp, Artificial Sequence
  source: /note="Description of Artificial Sequence: Synthetic oligonucleotide"
gcgacaggtgactgcagctgactacgacgtgatgtg

SEQ ID NO: 6 - DNA, 36 bp, Artificial Sequence
  source: /note="Description of Artificial Sequence: Synthetic oligonucleotide"
  modified_base (17)..(17): 2'-deoxyinosine
cacatcacgtcgtagtnagctgcagtcacctgtcgc

SEQ ID NO: 7 - DNA, 18 bp, Artificial Sequence
  source: /note="Description of Artificial Sequence: Synthetic oligonucleotide"
gctgcagtcacctgtcgc

SEQ ID NO: 8 - DNA, 19 bp, Artificial Sequence
  source: /note="Description of Artificial Sequence: Synthetic primer"
gcgacaggtgactgcagct

SEQ ID NO: 9 - DNA, 18 bp, Artificial Sequence
  source: /note="Description of Artificial Sequence: Synthetic oligonucleotide"
  modified_base (17)..(17): 2'-deoxyinosine
cacatcacgtcgtagtna

SEQ ID NO: 10 - DNA, 18 bp, Artificial Sequence
  source: /note="Description of Artificial Sequence: Synthetic primer"
gcgacaggtgactgcagc

SEQ ID NO: 11 - DNA, 36 bp, Artificial Sequence; identical to SEQ ID NO: 2
  source: /note="Description of Artificial Sequence: Synthetic oligonucleotide"
  modified_base (18)..(18): 2'-deoxyinosine

SEQ ID NO: 12 - DNA, 18 bp, Artificial Sequence
  source: /note="Description of Artificial Sequence: Synthetic oligonucleotide"
cgactacgacgtgatgtg

SEQ ID NO: 13 - DNA, 36 bp, Artificial Sequence; identical to SEQ ID NO: 2
  source: /note="Description of Artificial Sequence: Synthetic oligonucleotide"
  modified_base (18)..(18): Deoxyinosine

SEQ ID NO: 14 - DNA, 19 bp, Artificial Sequence
  source: /note="Description of Artificial Sequence: Synthetic primer"
gcgacaggtgactgcagct

SEQ ID NO: 15 - DNA, 36 bp, Artificial Sequence; identical to SEQ ID NO: 5
  source: /note="Description of Artificial Sequence: Synthetic oligonucleotide"

SEQ ID NO: 16 - DNA, 18 bp, Artificial Sequence
  source: /note="Description of Artificial Sequence: Synthetic oligonucleotide"
tgactacgacgtgatgtg

SEQ ID NO: 17 - DNA, 36 bp, Artificial Sequence; identical to SEQ ID NO: 6
  source: /note="Description of Artificial Sequence: Synthetic oligonucleotide"
  modified_base (17)..(17): 2'-deoxyinosine

SEQ ID NO: 18 - DNA, 18 bp, Artificial Sequence
  source: /note="Description of Artificial Sequence: Synthetic oligonucleotide"
gctgcagtcacctgtcgc

SEQ ID NO: 19 - DNA, 19 bp, Artificial Sequence
  source: /note="Description of Artificial Sequence: Synthetic primer"
gcgacaggtgactgcagct

SEQ ID NO: 20 - DNA, 18 bp, Artificial Sequence
  source: /note="Description of Artificial Sequence: Synthetic oligonucleotide"
  modified_base (17)..(17): 2'-deoxyinosine
cacatcacgtcgtagtna

SEQ ID NO: 21 - DNA, 17 bp, Artificial Sequence
  source: /note="Description of Artificial Sequence: Synthetic oligonucleotide"
cactacgacgtgatgtg

SEQ ID NO: 22 - DNA, 18 bp, Artificial Sequence
  source: /note="Description of Artificial Sequence: Synthetic primer"
gcgacaggtgactgcagc

SEQ ID NO: 23 - DNA, 37 bp, Artificial Sequence
  source: /note="Description of Artificial Sequence: Synthetic oligonucleotide"
  modified_base (18)..(18): 2'-deoxyinosine
cacatcacgtcgtagtcnagctgcagtcacctgtcgc

SEQ ID NO: 24 - DNA, 37 bp, Artificial Sequence
  source: /note="Description of Artificial Sequence: Synthetic oligonucleotide"
  modified_base (18)..(18): 2'-deoxyinosine
cacatcacgtcgtagtcnggctgcagtcacctgtcgc

SEQ ID NO: 25 - DNA, 37 bp, Artificial Sequence; identical to SEQ ID NO: 23
  source: /note="Description of Artificial Sequence: Synthetic oligonucleotide"
  modified_base (18)..(18): 2'-deoxyinosine

SEQ ID NO: 26 - DNA, 37 bp, Artificial Sequence; identical to SEQ ID NO: 23
  source: /note="Description of Artificial Sequence: Synthetic oligonucleotide"
  modified_base (18)..(18): 2'-deoxyinosine

SEQ ID NO: 27 - DNA, 19 bp, Artificial Sequence
  source: /note="Description of Artificial Sequence: Synthetic oligonucleotide"
tcgactacgacgtgatgtg

SEQ ID NO: 28 - DNA, 19 bp, Artificial Sequence
  source: /note="Description of Artificial Sequence: Synthetic oligonucleotide"
ccgactacgacgtgatgtg

SEQ ID NO: 29 - DNA, 19 bp, Artificial Sequence
  source: /note="Description of Artificial Sequence: Synthetic oligonucleotide"
acgactacgacgtgatgtg

SEQ ID NO: 30 - DNA, 19 bp, Artificial Sequence
  source: /note="Description of Artificial Sequence: Synthetic oligonucleotide"
gcgactacgacgtgatgtg

SEQ ID NO: 31 - DNA, 37 bp, Artificial Sequence; identical to SEQ ID NO: 23
  source: /note="Description of Artificial Sequence: Synthetic oligonucleotide"
  modified_base (18)..(18): Deoxyinosine

SEQ ID NO: 32 - DNA, 19 bp, Artificial Sequence
  source: /note="Description of Artificial Sequence: Synthetic primer"
gcgacaggtgactgcagct

SEQ ID NO: 33 - DNA, 36 bp, Artificial Sequence; identical to SEQ ID NO: 5
  source: /note="Description of Artificial Sequence: Synthetic oligonucleotide"

SEQ ID NO: 34 - DNA, 19 bp, Artificial Sequence
  source: /note="Description of Artificial Sequence: Synthetic oligonucleotide"
tcgactacgacgtgatgtg

SEQ ID NO: 35 - DNA, 18 bp, Artificial Sequence
  source: /note="Description of Artificial Sequence: Synthetic oligonucleotide"
gctgcagtcacctgtcgc

SEQ ID NO: 36 - DNA, 19 bp, Artificial Sequence
  source: /note="Description of Artificial Sequence: Synthetic primer"
gcgacaggtgactgcagct

SEQ ID NO: 37 - DNA, 19 bp, Artificial Sequence
  source: /note="Description of Artificial Sequence: Synthetic oligonucleotide"
  modified_base (17)..(17): 2'-deoxyinosine
cacatcacgtcgtagtnga

SEQ ID NO: 38 - DNA, 18 bp, Artificial Sequence
  source: /note="Description of Artificial Sequence: Synthetic oligonucleotide"
ccactacgacgtgatgtg

SEQ ID NO: 39 - DNA, 18 bp, Artificial Sequence
  source: /note="Description of Artificial Sequence: Synthetic primer"
gcgacaggtgactgcagc

SEQ ID NO: 40 - DNA, 36 bp, Artificial Sequence
  source: /note="Description of Artificial Sequence: Synthetic oligonucleotide"
cacatcacgtcgtagtcagctgcagtcacctgtcgc

SEQ ID NO: 41 - DNA, 36 bp, Artificial Sequence
  source: /note="Description of Artificial Sequence: Synthetic oligonucleotide"
cacatcacgtcgtagtcggctgcagtcacctgtcgc

SEQ ID NO: 42 - DNA, 36 bp, Artificial Sequence
  source: /note="Description of Artificial Sequence: Synthetic oligonucleotide"
cacatcacgtcgtagtctgctgcagtcacctgtcgc

SEQ ID NO: 43 - DNA, 36 bp, Artificial Sequence
  source: /note="Description of Artificial Sequence: Synthetic oligonucleotide"
cacatcacgtcgtagtccgctgcagtcacctgtcgc

SEQ ID NO: 44 - DNA, 78 bp, Artificial Sequence
  source: /note="Description of Artificial Sequence: Synthetic oligonucleotide"
  modified_base (36)..(36): 2'-deoxyinosine
  modified_base (58)..(58): Tamra-dT
tcgactacgacgtgacttttagtcacgtcgtagtcnagctgcagtcacctgctgcttnttgcagcaggtgactgcagc

SEQ ID NO: 45 - DNA, 79 bp, Artificial Sequence
  source: /note="Description of Artificial Sequence: Synthetic oligonucleotide"
  modified_base (36)..(36): 2'-deoxyinosine
  modified_base (58)..(58): Tamra-dT
tcgactacgacgtgacttttagtcacgtcgtagtcnagctgcagtcacctgctgcttnttgcagcaggtgactgcagct

SEQ ID NO: 46 - DNA, 42 bp, Artificial Sequence
  source: /note="Description of Artificial Sequence: Synthetic oligonucleotide"
  modified_base (21)..(21): Tamra-dT phosphate
gctgcagtcacctgctgcttnttgcagcaggtgactgcagct

SEQ ID NO: 47 - DNA, 38 bp, Artificial Sequence
  source: /note="Description of Artificial Sequence: Synthetic oligonucleotide"
  modified_base (36)..(36): 2'-deoxyinosine
ccgactacgacgtgacttttagtcacgtcgtagtcnga

SEQ ID NO: 48 - DNA, 78 bp, Artificial Sequence; identical to SEQ ID NO: 44
  source: /note="Description of Artificial Sequence: Synthetic oligonucleotide"
  modified_base (36)..(36): 2'-deoxyinosine
  modified_base (58)..(58): Tamra-dT

SEQ ID NO: 49 - DNA, 38 bp, Artificial Sequence; identical to SEQ ID NO: 47
  source: /note="Description of Artificial Sequence: Synthetic oligonucleotide"
  modified_base (36)..(36): 2'-deoxyinosine

SEQ ID NO: 50 - DNA, 58 bp, Artificial Sequence
  source: /note="Description of Artificial Sequence: Synthetic oligonucleotide"
  modified_base (16)..(16): 2'-deoxyinosine
  modified_base (38)..(38): Tamra-dT
agtcacgtcgtagtcnagctgcagtcacctgctgcttnttgcagcaggtgactgcagc

SEQ ID NO: 51 - DNA, 17 bp, Artificial Sequence
  source: /note="Description of Artificial Sequence: Synthetic oligonucleotide"
tcgactacgacgtgact

SEQ ID NO: 52 - DNA, 18 bp, Artificial Sequence
  source: /note="Description of Artificial Sequence: Synthetic oligonucleotide"
  modified_base (16)..(16): 2'-deoxyinosine
agtcacgtcgtagtcnga

SEQ ID NO: 53 - DNA, 17 bp, Artificial Sequence
  source: /note="Description of Artificial Sequence: Synthetic oligonucleotide"
ccgactacgacgtgact

SEQ ID NO: 54 - DNA, 78 bp, Artificial Sequence
  source: /note="Description of Artificial Sequence: Synthetic oligonucleotide"
  modified_base (35)..(35): 2'-deoxyinosine
  modified_base (57)..(57): Tamra-dT
cgactacgacgtgacttttagtcacgtcgtagtcnagctgcagtcacctgctgcttnttgcagcaggtgactgcagct

SEQ ID NO: 55 - DNA, 37 bp, Artificial Sequence
  source: /note="Description of Artificial Sequence: Synthetic oligonucleotide"
  modified_base (35)..(35): 2'-deoxyinosine
cgactacgacgtgacttttagtcacgtcgtagtcnaa

SEQ ID NO: 56 - DNA, 78 bp, Artificial Sequence
  source: /note="Description of Artificial Sequence: Synthetic oligonucleotide"
  modified_base (35)..(35): 2'-deoxyinosine
  modified_base (52)..(52): Tamra-dT
  modified_base (57)..(57): Biotin-dT
cgactacgacgtgacttttagtcacgtcgtagtcnagctgcagtcacctgcngcttnttgcagcaggtgactgcagct

SEQ ID NO: 57 - DNA, 38 bp, Artificial Sequence; identical to SEQ ID NO: 47
  source: /note="Description of Artificial Sequence: Synthetic oligonucleotide"
  modified_base (36)..(36): 2'-deoxyinosine

SEQ ID NO: 58 - DNA, 62 bp, Artificial Sequence
  source: /note="Description of Artificial Sequence: Synthetic oligonucleotide"
  modified_base (60)..(60): 2'-deoxyinosine
acgagtgacctggttttttttttttttttttttttttttttttttttaccaggtcactcntg

SEQ ID NO: 59 - DNA, 58 bp, Artificial Sequence
  source: /note="Description of Artificial Sequence: Synthetic oligonucleotide"
  modified_base (16)..(16): 2'-deoxyinosine
  modified_base (33)..(33): Tamra-dT
  modified_base (38)..(38): Biotin-dT
agtcacgtcgtagtcnagctgcagtcacctgcngcttnttgcagcaggtgactgcagc

SEQ ID NO: 60 - DNA, 18 bp, Artificial Sequence
  source: /note="Description of Artificial Sequence: Synthetic oligonucleotide"
  modified_base (16)..(16): 2'-deoxyinosine
agtcacgtcgtagtcnaa

SEQ ID NO: 61 - DNA, 67 bp, Artificial Sequence
  source: /note="Description of Artificial Sequence: Synthetic oligonucleotide"
  modified_base (16)..(16): 2'-deoxyinosine
agtcacgtcgtagtcnagctgcagtcacctgctgcttttttttttttttgcagcaggtgactgcagc

SEQ ID NO: 62 - DNA, 67 bp, Artificial Sequence; identical to SEQ ID NO: 61
  source: /note="Description of Artificial Sequence: Synthetic oligonucleotide"
  modified_base (16)..(16): 2'-deoxyinosine

SEQ ID NO: 63 - DNA, 58 bp, Artificial Sequence
  source: /note="Description of Artificial Sequence: Synthetic oligonucleotide"
  modified_base (16)..(16): 2'-deoxyinosine
  modified_base (38)..(38): 5''-thiophosphate-Sp9-Sp9-Sp9-5-methylC
agtcacgtcgtagtcnagctgcagtcacctgctgcttcttgcagcaggtgactgcagc

SEQ ID NO: 64 - DNA, 58 bp, Artificial Sequence; identical to SEQ ID NO: 63
  source: /note="Description of Artificial Sequence: Synthetic oligonucleotide"
  modified_base (16)..(16): 2'-deoxyinosine
  modified_base (38)..(38): 5''-phosphate-Sp9-Sp9-Sp9-5-methylC

SEQ ID NO: 65 - DNA, 59 bp, Artificial Sequence
  source: /note="Description of Artificial Sequence: Synthetic oligonucleotide"
  modified_base (16)..(16): 2'-deoxyinosine
  modified_base (38)..(38): 5''-thiophosphate-Sp9-Sp9-Sp9-5-methylC
agtcacgtcgtagtcnagctgcagtcacctgctgcttcttgcagcaggtgactgcagct

SEQ ID NO: 66 - DNA, 59 bp, Artificial Sequence
  source: /note="Description of Artificial Sequence: Synthetic oligonucleotide"
  modified_base (38)..(38): 5''-thiophosphate-Sp9-Sp9-Sp9-5-methylC
agtcacgtcgtagtcgagctgcagtcacctgctgcttcttgcagcaggtgactgcagct

SEQ ID NO: 67 - DNA, 18 bp, Artificial Sequence
  source: /note="Description of Artificial Sequence: Synthetic oligonucleotide"
  modified_base (16)..(16): 2'-deoxyinosine
agtcacgtcgtagtcnaa

SEQ ID NO: 68 - DNA, 18 bp, Artificial Sequence
  primer sequence - figure 51
gcgacaggtgactgcagc

SEQ ID NO: 69 - DNA, 18 bp, Artificial Sequence
  template sequence - figure 51
gctgcagtcacctgtcgc